European Patent Specification EP 3 768 429 B1, published January 1, 2025. Title: MEMORY WRITING. Applicant: IMEC VZW. The sequence listing filed with the application follows.

SEQUENCE LISTING (2 sequences)

SEQ ID NO: 1 - DNA, 4 bp, Artificial Sequence
  Example of strand of memory writing substrate DNA
gtac

SEQ ID NO: 2 - DNA, 13 bp, Artificial Sequence
  Example of strand of memory writing substrate DNA
aggctgctactct